European Patent Specification EP 3 625 366 B1, published February 19, 2025. Title: Single nucleotide detection method and associated probes. Applicant: Base4 Innovation Limited. The sequence listing filed with the application follows.

SEQUENCE LISTING (3 sequences)

SEQ ID NO: 1 - DNA, 61 bp, Artificial sequence
  single-stranded first oligonucleotide 1
  T labelled with Atto 700 dye (33)..(34): F represents a deoxythymidine nucleotide (T) labelled with Atto 700 dye
  T labelled with a BHQ-2 quencher (35)..(35): Q represents a deoxythymidine nucleotide labelled with a BHQ-2 quencher
  inverted 3' dT nucleotide (61)..(61): X represents an inverted 3' dT nucleotide
gctgtgccgggctcgtgtctctgcgtttcttgtttgtgtgcattgcataggttcacgatat

SEQ ID NO: 2 - DNA, 15 bp, Artificial sequence
  single-stranded oligonucleotide 2
cgtgaacctatgcaa

SEQ ID NO: 3 - DNA, 21 bp, Artificial sequence
  single-stranded oligonucleotide 3
  5' phosphate group (1)..(1): 5' phosphate group
  3' inverted dT nucleotide (21)..(21): X represents 3' inverted dT nucleotide
gcgaacgtaaaatgtcatggt